European Patent Specification EP 3 351 632 B1, published July 16, 2025. Title: Structurally reinforced miRNA inhibitor S-TuD. Applicant: THE UNIVERSITY OF TOKYO GENE DESIGN INC. The sequence listing filed with the application follows.

SEQUENCE LISTING (80 sequences)

SEQ ID NO: 1 - DNA, 52 bp, artificial sequence
  original sense sequence
  2'-OMe (1)..(52)
gacggcgcuaggaucaucaaacaaugugcagacuacuguaaaguauucuggu

SEQ ID NO: 2 - DNA, 52 bp, artificial sequence
  original antisense sequence
  2'-OMe (1)..(52)
cugccgcgauccuaguagaaaugucaucagacguguaacaaacauaagacca

SEQ ID NO: 3 - DNA, 52 bp, artificial sequence; identical to SEQ ID NO: 1
  sense sequence (1)
  2'-OMe (1)..(2)
  2'-F (3)..(3)
  2'-OMe (4)..(5)
  2'-F (6)..(6)
  2'-OMe (7)..(7)
  2'-F (8)..(9)
  2'-OMe (10)..(13)
  2'-F (14)..(15)
  2'-OMe (16)..(16)
  2'-F (17)..(18)
  2'-OMe (19)..(21)
  2'-F (22)..(22)
  2'-OMe (23)..(24)
  2'-F (25)..(25)
  2'-OMe (26)..(26)
  2'-F (27)..(27)
  2'-OMe (28)..(28)
  2'-F (29)..(29)
  2'-OMe (30)..(32)
  2'-F (33)..(34)
  2'-OMe (35)..(35)
  2'-F (36)..(37)
  2'-OMe (38)..(38)
  2'-F (39)..(39)
  2'-OMe (40)..(43)
  2'-F (44)..(44)
  2'-OMe (45)..(45)
  2'-F (46)..(49)
  2'-OMe (50)..(51)
  2'-F (52)..(52)

SEQ ID NO: 4 - DNA, 52 bp, artificial sequence; identical to SEQ ID NO: 2
  antisense sequence (1)
  2'-F (1)..(2)
  2'-OMe (3)..(3)
  2'-F (4)..(5)
  2'-OMe (6)..(6)
  2'-F (7)..(7)
  2'-OMe (8)..(9)
  2'-F (10)..(13)
  2'-OMe (14)..(15)
  2'-F (16)..(16)
  2'-OMe (17)..(21)
  2'-F (22)..(22)
  2'-OMe (23)..(23)
  2'-F (24)..(25)
  2'-OMe (26)..(26)
  2'-F (27)..(28)
  2'-OMe (29)..(31)
  2'-F (32)..(32)
  2'-OMe (33)..(33)
  2'-F (34)..(34)
  2'-OMe (35)..(35)
  2'-F (36)..(36)
  2'-OMe (37)..(38)
  2'-F (39)..(39)
  2'-OMe (40)..(42)
  2'-F (43)..(43)
  2'-OMe (44)..(44)
  2'-F (45)..(45)
  2'-OMe (46)..(49)
  2'-F (50)..(51)
  2'-OMe (52)..(52)

SEQ ID NO: 5 - DNA, 52 bp, artificial sequence
  sense sequence (2)
  2'-OMe (1)..(8)
  BNANC(NMe) (9)..(9)
  2'-OMe (10)..(13)
  BNANC(NMe) (14)..(14)
  2'-OMe (15)..(46)
  BNANC(NMe) (47)..(47)
  2'-OMe (48)..(51)
  BNANC(NMe) (52)..(52)
gacggcgctaggatcaucaaacaaugugcagacuacuguaaaguautcuggt

SEQ ID NO: 6 - DNA, 52 bp, artificial sequence; identical to SEQ ID NO: 2
  antisense sequence (2)
  2'-OMe (1)..(52)

SEQ ID NO: 7 - DNA, 52 bp, artificial sequence
  sense sequence (3)
  2'-OMe (1)..(8)
  BNANC(NMe) (9)..(9)
  2'-OMe (10)..(51)
  BNANC(NMe) (52)..(52)
gacggcgctaggaucaucaaacaaugugcagacuacuguaaaguauucuggt

SEQ ID NO: 8 - DNA, 52 bp, artificial sequence
  antisense sequence (3)
  2'-OMe (1)..(12)
  BNANC(NMe) (13)..(13)
  2'-OMe (14)..(44)
  BNANC(NMe) (45)..(45)
  2'-OMe (46)..(52)
cugccgcgaucctaguagaaaugucaucagacguguaacaaacataagacca

SEQ ID NO: 9 - DNA, 52 bp, artificial sequence; identical to SEQ ID NO: 5
  sense sequence (4)
  2'-OMe (1)..(8)
  BNANC(NMe) (9)..(9)
  2'-OMe (10)..(13)
  BNANC(NMe) (14)..(14)
  2'-OMe (15)..(46)
  BNANC(NMe) (47)..(47)
  2'-OMe (48)..(51)
  BNANC(NMe) (52)..(52)

SEQ ID NO: 10 - DNA, 52 bp, artificial sequence; identical to SEQ ID NO: 2
  antisense sequence (4)
  2'-OMe (1)..(8)
  BNANC(NMe) (9)..(9)
  2'-OMe (10)..(13)
  BNANC(NMe) (14)..(14)
  2'-OMe (15)..(46)
  BNANC(NMe) (47)..(47)
  2'-OMe (48)..(51)
  BNANC(NMe) (52)..(52)

SEQ ID NO: 11 - DNA, 44 bp, artificial sequence
  sense sequence (5)
  BNANC(NMe) (1)..(1)
  2'-OMe (2)..(5)
  BNANC(NMe) (6)..(6)
  2'-OMe (7)..(38)
  BNANC(NMe) (39)..(39)
  2'-OMe (40)..(43)
  BNANC(NMe) (44)..(44)
taggatcaucaaacaaugugcagacuacuguaaaguautcuggt

SEQ ID NO: 12 - DNA, 44 bp, artificial sequence
  antisense sequence (5)
  BNANC(NMe) (1)..(1)
  2'-OMe (2)..(5)
  BNANC(NMe) (6)..(6)
  2'-OMe (7)..(38)
  BNANC(NMe) (39)..(39)
  2'-OMe (40)..(43)
  BNANC(NMe) (44)..(44)
auccuaguagaaaugucaucagacguguaacaaacauaagacca

SEQ ID NO: 13 - DNA, 52 bp, artificial sequence
  sense sequence (16)
  BNANC(NMe) (1)..(1)
  2'-OMe (1)..(1)
  2'-OMe (2)..(43)
  BNANC(NMe) (44)..(44)
  2'-OMe (45)..(48)
  BNANC(NMe) (49)..(49)
  2'-OMe (50)..(52)
tacggcgcuaggaucaucaaacaaugugcagacuacuguaaagtauuctgga

SEQ ID NO: 14 - DNA, 52 bp, artificial sequence
  antisense sequence (16)
  2'-OMe (1)..(9)
  BNANC(NMe) (10)..(10)
  2'-OMe (11)..(15)
  BNANC(NMe) (16)..(16)
  2'-OMe (17)..(51)
  BNANC(NMe) (52)..(52)
augccgcgatccuagtagaaaugucaucagacguguaacaaacauaagacct

SEQ ID NO: 15 - DNA, 52 bp, artificial sequence
  sense sequence (22)
  BNANC(NMe) (1)..(1)
  2'-OMe (2)..(33)
  BNANC(NMe) (34)..(34)
  2'-OMe (35)..(36)
  BNANC(NMe) (37)..(37)
  2'-OMe (38)..(43)
  BNANC(NMe) (44)..(44)
  2'-OMe (45)..(48)
  BNANC(NMe) (49)..(49)
  2'-OMe (50)..(52)
tacggcgcuaggaucaucaaacaaugugcagactactguaaagtauuctgga

SEQ ID NO: 16 - DNA, 52 bp, artificial sequence
  antisense sequence (22)
  2'-OMe (1)..(9)
  BNANC(NMe) (10)..(10)
  2'-OMe (11)..(15)
  BNANC(NMe) (16)..(16)
  2'-OMe (17)..(23)
  BNANC(NMe) (24)..(24)
  2'-OMe (25)..(26)
  BNANC(NMe) (27)..(27)
  2'-OMe (28)..(51)
  BNANC(NMe) (52)..(52)
augccgcgatccuagtagaaaugtcatcagacguguaacaaacauaagacct

SEQ ID NO: 17 - DNA, 52 bp, artificial sequence
  sense sequence (23)
  BNANC(NMe) (1)..(1)
  2'-OMe (2)..(23)
  BNANC(NMe) (24)..(24)
  2'-OMe (25)..(26)
  BNANC(NMe) (27)..(27)
  2'-OMe (28)..(43)
  BNANC(NMe) (44)..(44)
  2'-OMe (45)..(48)
  BNANC(NMe) (49)..(49)
  2'-OMe (50)..(52)
tacggcgcuaggaucaucaaacaaugtgcagacuacuguaaagtauuctgga

SEQ ID NO: 18 - DNA, 52 bp, artificial sequence
  antisense sequence (23)
  2'-OMe (1)..(9)
  BNANC(NMe) (10)..(10)
  2'-OMe (11)..(15)
  BNANC(NMe) (16)..(16)
  2'-OMe (17)..(33)
  BNANC(NMe) (34)..(34)
  2'-OMe (35)..(36)
  BNANC(NMe) (37)..(37)
  2'-OMe (38)..(51)
  BNANC(NMe) (52)..(52)
augccgcgatccuagtagaaaugucaucagacgtguaacaaacauaagacct

SEQ ID NO: 19 - DNA, 52 bp, artificial sequence
  sense sequence (24)
  2'-OMe (1)..(1)
  BNANC(NMe) (2)..(2)
  2'-OMe (3)..(23)
  BNANC(NMe) (24)..(24)
  2'-OMe (25)..(26)
  BNANC(NMe) (27)..(27)
  2'-OMe (28)..(43)
  BNANC(NMe) (44)..(44)
  2'-OMe (45)..(51)
  BNANC(NMe) (52)..(52)
atcggcgcuaggaucaucaaacaaugtgcagacuacuguaaagtauucugat

SEQ ID NO: 20 - DNA, 52 bp, artificial sequence
  antisense sequence (24)
  BNANC(NMe) (1)..(1)
  2'-OMe (2)..(9)
  BNANC(NMe) (10)..(10)
  2'-OMe (11)..(33)
  BNANC(NMe) (34)..(34)
  2'-OMe (35)..(36)
  BNANC(NMe) (37)..(37)
  2'-OMe (38)..(50)
  BNANC(NMe) (51)..(51)
  2'-OMe (52)..(52)
tagccgcgatccuaguagaaaugucaucagacgtguaacaaacauaagacta

SEQ ID NO: 21 - DNA, 44 bp, artificial sequence
  sense sequence (17)
  BNANC(NMe) (1)..(1)
  2'-OMe (2)..(25)
  BNANC(NMe) (26)..(26)
  2'-OMe (27)..(28)
  BNANC(NMe) (29)..(29)
  2'-OMe (30)..(38)
  BNANC(NMe) (39)..(39)
  2'-OMe (40)..(43)
  BNANC(NMe) (44)..(44)
taggaucaucaaacaaugugcagactactguaaaguautcuggt

SEQ ID NO: 22 - DNA, 44 bp, artificial sequence
  antisense sequence (17)
  2'-OMe (1)..(4)
  BNANC(NMe) (5)..(5)
  2'-OMe (6)..(7)
  BNANC(NMe) (8)..(8)
  2'-OMe (9)..(15)
  BNANC(NMe) (16)..(16)
  2'-OMe (17)..(18)
  BNANC(NMe) (19)..(19)
  2'-OMe (20)..(36)
  BNANC(NMe) (37)..(37)
  2'-OMe (38)..(44)
aucctagtagaaaugtcatcagacguguaacaaacataagacca

SEQ ID NO: 23 - DNA, 44 bp, artificial sequence
  sense sequence (18)
  BNANC(NMe) (1)..(1)
  2'-OMe (2)..(15)
  BNANC(NMe) (16)..(16)
  2'-OMe (17)..(18)
  BNANC(NMe) (19)..(19)
  2'-OMe (20)..(38)
  BNANC(NMe) (39)..(39)
  2'-OMe (40)..(43)
  BNANC(NMe) (44)..(44)
taggaucaucaaacaaugtgcagacuacuguaaaguautcuggt

SEQ ID NO: 24 - DNA, 44 bp, artificial sequence
  antisense sequence (18)
  2'-OMe (1)..(4)
  BNANC(NMe) (5)..(5)
  2'-OMe (6)..(7)
  BNANC(NMe) (8)..(8)
  2'-OMe (9)..(25)
  BNANC(NMe) (26)..(26)
  2'-OMe (27)..(28)
  BNANC(NMe) (29)..(29)
  2'-OMe (30)..(36)
  BNANC(NMe) (37)..(37)
  2'-OMe (38)..(44)
aucctagtagaaaugucaucagacgtguaacaaacataagacca

SEQ ID NO: 25 - DNA, 52 bp, artificial sequence; identical to SEQ ID NO: 17
  sense sequence (23)-(1)
  BNANC(NMe) (1)..(1)
  2'-OMe (2)..(23)
  phosphorothioate linkage (19)..(41)
  BNANC(NMe) (24)..(24)
  2'-OMe (25)..(26)
  BNANC(NMe) (27)..(27)
  2'-OMe (28)..(43)
  BNANC(NMe) (44)..(44)
  2'-OMe (45)..(48)
  BNANC(NMe) (49)..(49)
  2'-OMe (50)..(52)

SEQ ID NO: 26 - DNA, 52 bp, artificial sequence; identical to SEQ ID NO: 18
  antisense sequence (23)-(1)
  2'-OMe (1)..(9)
  BNANC(NMe) (10)..(10)
  2'-OMe (11)..(15)
  BNANC(NMe) (16)..(16)
  2'-OMe (17)..(33)
  phosphorothioate linkage (19)..(41)
  BNANC(NMe) (34)..(34)
  2'-OMe (35)..(36)
  BNANC(NMe) (37)..(37)
  2'-OMe (38)..(51)
  BNANC(NMe) (52)..(52)

SEQ ID NO: 27 - DNA, 52 bp, artificial sequence; identical to SEQ ID NO: 17
  sense sequence (23)-(2)
  phosphorothioate linkage (1)..(17)
  BNANC(NMe) (1)..(1)
  2'-OMe (2)..(23)
  BNANC(NMe) (24)..(24)
  2'-OMe (25)..(26)
  BNANC(NMe) (27)..(27)
  2'-OMe (28)..(43)
  phosphorothioate linkage (43)..(51)
  BNANC(NMe) (44)..(44)
  2'-OMe (45)..(48)
  BNANC(NMe) (49)..(49)
  2'-OMe (50)..(52)

SEQ ID NO: 28 - DNA, 52 bp, artificial sequence; identical to SEQ ID NO: 18
  antisense sequence (23)-(2)
  phosphorothioate linkage (1)..(17)
  2'-OMe (1)..(9)
  BNANC(NMe) (10)..(10)
  2'-OMe (11)..(15)
  BNANC(NMe) (16)..(16)
  2'-OMe (17)..(33)
  BNANC(NMe) (34)..(34)
  2'-OMe (35)..(36)
  BNANC(NMe) (37)..(37)
  2'-OMe (38)..(51)
  phosphorothioate linkage (43)..(51)
  BNANC(NMe) (52)..(52)

SEQ ID NO: 29 - DNA, 52 bp, artificial sequence; identical to SEQ ID NO: 17
  sense sequence (23)-(3)
  BNANC(NMe) (1)..(1)
  phosphorothioate linkage (1)..(51)
  2'-OMe (2)..(23)
  BNANC(NMe) (24)..(24)
  2'-OMe (25)..(26)
  BNANC(NMe) (27)..(27)
  2'-OMe (28)..(43)
  BNANC(NMe) (44)..(44)
  2'-OMe (45)..(48)
  BNANC(NMe) (49)..(49)
  2'-OMe (50)..(52)

SEQ ID NO: 30 - DNA, 52 bp, artificial sequence; identical to SEQ ID NO: 18
  antisense sequence (23)-(3)
  phosphorothioate linkage (1)..(51)
  2'-OMe (1)..(9)
  BNANC(NMe) (10)..(10)
  2'-OMe (11)..(15)
  BNANC(NMe) (16)..(16)
  2'-OMe (17)..(33)
  BNANC(NMe) (34)..(34)
  2'-OMe (35)..(36)
  BNANC(NMe) (37)..(37)
  2'-OMe (38)..(51)
  BNANC(NMe) (52)..(52)

SEQ ID NO: 31 - DNA, 44 bp, artificial sequence
  sense sequence (1)'
  2'-OMe (1)..(44)
uaggaucaucaaacaaugugcagacuacuguaaaguauucuggu

SEQ ID NO: 32 - DNA, 44 bp, artificial sequence; identical to SEQ ID NO: 12
  antisense sequence (1)'
  2'-OMe (1)..(44)

SEQ ID NO: 33 - DNA, 44 bp, artificial sequence
  sense sequence (6)'
  BNANC(NMe) (1)..(1)
  2'-OMe (2)..(38)
  BNANC(NMe) (39)..(39)
  2'-OMe (40)..(43)
  BNANC(NMe) (44)..(44)
taggaucaucaaacaaugugcagacuacuguaaaguautcuggt

SEQ ID NO: 34 - DNA, 44 bp, artificial sequence
  antisense sequence (6)'
  2'-OMe (1)..(4)
  BNANC(NMe) (5)..(5)
  2'-OMe (6)..(7)
  BNANC(NMe) (8)..(8)
  2'-OMe (9)..(36)
  BNANC(NMe) (37)..(37)
  2'-OMe (38)..(44)
aucctagtagaaaugucaucagacguguaacaaacataagacca

SEQ ID NO: 35 - DNA, 52 bp, artificial sequence; identical to SEQ ID NO: 17
  sense sequence (23)
  BNANC(NMe) (1)..(1)
  2'-OMe (2)..(23)
  BNANC(NMe) (24)..(24)
  2'-OMe (25)..(26)
  BNANC(NMe) (27)..(27)
  2'-OMe (28)..(43)
  BNANC(NMe) (44)..(44)
  2'-OMe (45)..(48)
  BNANC(NMe) (49)..(49)
  2'-OMe (50)..(52)

SEQ ID NO: 36 - DNA, 52 bp, artificial sequence; identical to SEQ ID NO: 18
  antisense sequence (23)
  2'-OMe (1)..(9)
  BNANC(NMe) (10)..(10)
  2'-OMe (11)..(15)
  BNANC(NMe) (16)..(16)
  2'-OMe (17)..(33)
  BNANC(NMe) (34)..(34)
  2'-OMe (35)..(36)
  BNANC(NMe) (37)..(37)
  2'-OMe (38)..(51)
  BNANC(NMe) (52)..(52)

SEQ ID NO: 37 - DNA, 56 bp, artificial sequence
  sense sequence (41)
  2'-OMe (1)..(56)
uacggcgcuaggaucaucaacccaucauuacccggcaguauuacaaguauucugga

SEQ ID NO: 38 - DNA, 56 bp, artificial sequence
  antisense sequence (41)
  2'-OMe (1)..(56)
augccgcgauccuaguagaacauuaugacggcccauuacuacccaacauaagaccu

SEQ ID NO: 39 - DNA, 56 bp, artificial sequence
  sense sequence (42)
  BNANC(NMe) (1)..(1)
  2'-OMe (2)..(47)
  BNANC(NMe) (48)..(48)
  2'-OMe (49)..(52)
  BNANC(NMe) (53)..(53)
  2'-OMe (54)..(56)
tacggcgcuaggaucaucaacccaucauuacccggcaguauuacaagtauuctgga

SEQ ID NO: 40 - DNA, 56 bp, artificial sequence
  antisense sequence (42)
  2'-OMe (1)..(9)
  BNANC(NMe) (10)..(10)
  2'-OMe (11)..(15)
  BNANC(NMe) (16)..(16)
  2'-OMe (17)..(55)
  BNANC(NMe) (56)..(56)
augccgcgatccuagtagaacauuaugacggcccauuacuacccaacauaagacct

SEQ ID NO: 41 - DNA, 56 bp, artificial sequence
  sense sequence (43)
  BNANC(NMe) (1)..(1)
  2'-OMe (2)..(38)
  BNANC(NMe) (39)..(39)
  2'-OMe (40)..(41)
  BNANC(NMe) (42)..(42)
  2'-OMe (43)..(47)
  BNANC(NMe) (48)..(48)
  2'-OMe (49)..(52)
  BNANC(NMe) (53)..(53)
  2'-OMe (54)..(56)
tacggcgcuaggaucaucaacccaucauuacccggcagtautacaagtauuctgga

SEQ ID NO: 42 - DNA, 56 bp, artificial sequence
  antisense sequence (43)
  2'-OMe (1)..(9)
  BNANC(NMe) (10)..(10)
  2'-OMe (11)..(15)
  BNANC(NMe) (16)..(16)
  2'-OMe (17)..(22)
  BNANC(NMe) (23)..(23)
  2'-OMe (24)..(25)
  BNANC(NMe) (26)..(26)
  2'-OMe (27)..(55)
  BNANC(NMe) (56)..(56)
augccgcgatccuagtagaacatuatgacggcccauuacuacccaacauaagacct

SEQ ID NO: 43 - DNA, 56 bp, artificial sequence
  sense sequence (44)
  BNANC(NMe) (1)..(1)
  2'-OMe (2)..(27)
  BNANC(NMe) (28)..(28)
  2'-OMe (29)..(30)
  BNANC(NMe) (31)..(31)
  2'-OMe (32)..(47)
  BNANC(NMe) (48)..(48)
  2'-OMe (49)..(52)
  BNANC(NMe) (53)..(53)
  2'-OMe (54)..(56)
tacggcgcuaggaucaucaacccaucatuacccggcaguauuacaagtauuctgga

SEQ ID NO: 44 - DNA, 56 bp, artificial sequence
  antisense sequence (44)
  2'-OMe (1)..(9)
  BNANC(NMe) (10)..(10)
  2'-OMe (11)..(15)
  BNANC(NMe) (16)..(16)
  2'-OMe (17)..(33)
  BNANC(NMe) (34)..(34)
  2'-OMe (35)..(36)
  BNANC(NMe) (37)..(37)
  2'-OMe (38)..(55)
  BNANC(NMe) (56)..(56)
augccgcgatccuagtagaacauuaugacggcccautacuacccaacauaagacct

SEQ ID NO: 45 - DNA, 48 bp, artificial sequence
  sense sequence (45)
  BNANC(NMe) (1)..(1)
  2'-OMe (2)..(19)
  BNANC(NMe) (20)..(20)
  2'-OMe (21)..(22)
  BNANC(NMe) (23)..(23)
  2'-OMe (24)..(42)
  BNANC(NMe) (43)..(43)
  2'-OMe (44)..(47)
  BNANC(NMe) (48)..(48)
taggaucaucaacccaucatuacccggcaguauuacaaguautcuggt

SEQ ID NO: 46 - DNA, 48 bp, artificial sequence
  antisense sequence (45)
  2'-OMe (1)..(4)
  BNANC(NMe) (5)..(5)
  2'-OMe (6)..(7)
  BNANC(NMe) (8)..(8)
  2'-OMe (9)..(25)
  BNANC(NMe) (26)..(26)
  2'-OMe (27)..(28)
  BNANC(NMe) (29)..(29)
  2'-OMe (30)..(40)
  BNANC(NMe) (41)..(41)
  2'-OMe (42)..(48)
aucctagtagaacauuaugacggcccautacuacccaacataagacca

SEQ ID NO: 47 - DNA, 51 bp, artificial sequence
  sense sequence (51)
  2'-OMe (1)..(51)
uacggcgcuaggaucaucaacaucagucggauaagcuacaaguauucugga

SEQ ID NO: 48 - DNA, 51 bp, artificial sequence
  antisense sequence (51)
  2'-OMe (1)..(51)
augccgcgauccuaguagaacaucgaauaggcugacuacaacauaagaccu

SEQ ID NO: 49 - DNA, 51 bp, artificial sequence
  sense sequence (52)
  BNANC(NMe) (1)..(1)
  2'-OMe (2)..(42)
  BNANC(NMe) (43)..(43)
  2'-OMe (44)..(47)
  BNANC(NMe) (48)..(48)
  2'-OMe (49)..(51)
tacggcgcuaggaucaucaacaucagucggauaagcuacaagtauuctgga

SEQ ID NO: 50 - DNA, 51 bp, artificial sequence
  antisense sequence (52)
  2'-OMe (1)..(9)
  BNANC(NMe) (10)..(10)
  2'-OMe (11)..(15)
  BNANC(NMe) (16)..(16)
  2'-OMe (17)..(50)
  BNANC(NMe) (51)..(51)
augccgcgatccuagtagaacaucgaauaggcugacuacaacauaagacct

SEQ ID NO: 51 - DNA, 51 bp, artificial sequence; identical to SEQ ID NO: 49
  sense sequence (53)
  BNANC(NMe) (1)..(1)
  2'-OMe (2)..(22)
  BNANC(NMe) (23)..(23)
  2'-OMe (24)..(25)
  BNANC(NMe) (26)..(26)
  2'-OMe (27)..(42)
  BNANC(NMe) (43)..(43)
  2'-OMe (44)..(47)
  BNANC(NMe) (48)..(48)
  2'-OMe (49)..(51)

SEQ ID NO: 52 - DNA, 51 bp, artificial sequence; identical to SEQ ID NO: 50
  antisense sequence (53)
  2'-OMe (1)..(9)
  BNANC(NMe) (10)..(10)
  2'-OMe (11)..(15)
  BNANC(NMe) (16)..(16)
  2'-OMe (17)..(33)
  BNANC(NMe) (34)..(34)
  2'-OMe (35)..(36)
  BNANC(NMe) (37)..(37)
  2'-OMe (38)..(50)
  BNANC(NMe) (51)..(51)

SEQ ID NO: 53 - DNA, 43 bp, artificial sequence
  sense sequence (54)
  BNANC(NMe) (1)..(1)
  2'-OMe (2)..(37)
  BNANC(NMe) (38)..(38)
  2'-OMe (39)..(42)
  BNANC(NMe) (43)..(43)
taggaucaucaacaucagucggauaagcuacaaguautcuggt

SEQ ID NO: 54 - DNA, 43 bp, artificial sequence
  antisense sequence (54)
  2'-OMe (1)..(4)
  BNANC(NMe) (5)..(5)
  2'-OMe (6)..(7)
  BNANC(NMe) (8)..(8)
  2'-OMe (9)..(35)
  BNANC(NMe) (36)..(36)
  2'-OMe (37)..(43)
aucctagtagaacaucgaauaggcugacuacaacataagacca

SEQ ID NO: 55 - DNA, 43 bp, artificial sequence; identical to SEQ ID NO: 53
  sense sequence (55)
  BNANC(NMe) (1)..(1)
  2'-OMe (2)..(14)
  BNANC(NMe) (15)..(15)
  2'-OMe (16)..(17)
  BNANC(NMe) (18)..(18)
  2'-OMe (19)..(37)
  BNANC(NMe) (38)..(38)
  2'-OMe (39)..(42)
  BNANC(NMe) (43)..(43)

SEQ ID NO: 56 - DNA, 43 bp, artificial sequence; identical to SEQ ID NO: 54
  antisense sequence (55)
  2'-OMe (1)..(4)
  BNANC(NMe) (5)..(5)
  2'-OMe (6)..(7)
  BNANC(NMe) (8)..(8)
  2'-OMe (9)..(25)
  BNANC(NMe) (26)..(26)
  2'-OMe (27)..(28)
  BNANC(NMe) (29)..(29)
  2'-OMe (30)..(35)
  BNANC(NMe) (36)..(36)
  2'-OMe (37)..(43)

SEQ ID NO: 57 - DNA, 59 bp, artificial sequence
  sense sequence of S-TuD NC2
  2'-OMe (1)..(59)
gacggcgcuaggaucaucaacuaucgcgaguaucgacgucgaggcccaaguauucuggu

SEQ ID NO: 58 - DNA, 59 bp, artificial sequence
  antisense sequence of S-TuD NC2
  2'-OMe (1)..(59)
cugccgcgauccuaguagaacccggagcugcagcuaugagcgcuaucaacauaagacca

SEQ ID NO: 59 - DNA, 44 bp, artificial sequence
  sense sequence (2)'
  BNANC(NMe) (1)..(1)
  2'-OMe (2)..(5)
  BNANC(NMe) (6)..(6)
  2'-OMe (7)..(38)
  BNANC(NMe) (39)..(39)
  2'-OMe (40)..(40)
  2'-OMe (40)..(43)
  2'-OMe (42)..(43)
  BNANC(NMe) (42)..(43)
  BNANC(NMe) (44)..(44)
taggatcaucaaacaaugugcagacuacuguaaaguautctggt

SEQ ID NO: 60 - DNA, 44 bp, artificial sequence
  antisense sequence (2)'
  2'-OMe (1)..(1)
  BNANC(NMe) (2)..(2)
  2'-OMe (3)..(7)
  BNANC(NMe) (8)..(8)
  2'-OMe (9)..(36)
  BNANC(NMe) (37)..(37)
  2'-OMe (38)..(44)
atccuagtagaaaugucaucagacguguaacaaacataagacca

SEQ ID NO: 61 - DNA, 44 bp, artificial sequence; identical to SEQ ID NO: 33
  sense sequence (7)'
  LNA (1)..(1)
  2'-OMe (2)..(38)
  LNA (39)..(39)
  2'-OMe (40)..(43)
  LNA (44)..(44)

SEQ ID NO: 62 - DNA, 44 bp, artificial sequence; identical to SEQ ID NO: 34
  antisense sequence (7)'
  2'-OMe (1)..(4)
  LNA (5)..(5)
  2'-OMe (6)..(7)
  LNA (8)..(8)
  2'-OMe (9)..(36)
  LNA (37)..(37)
  2'-OMe (38)..(44)

SEQ ID NO: 63 - DNA, 44 bp, artificial sequence
  sense sequence (8)'
  BNANC(NMe) (1)..(1)
  2'-OMe (2)..(5)
  BNANC(NMe) (6)..(6)
  2'-OMe (7)..(8)
  BNANC(NMe) (9)..(9)
  2'-OMe (10)..(35)
  BNANC(NMe) (36)..(36)
  2'-OMe (37)..(37)
  BNANC(NMe) (38)..(38)
  BNANC(NMe) (39)..(39)
  2'-OMe (40)..(40)
  BNANC(NMe) (41)..(41)
  2'-OMe (42)..(43)
  BNANC(NMe) (44)..(44)
taggatcatcaaacaaugugcagacuacuguaaagtattctggt

SEQ ID NO: 64 - DNA, 44 bp, artificial sequence
  antisense sequence (8)'
  2'-OMe (1)..(1)
  BNANC(NMe) (2)..(2)
  2'-OMe (3)..(4)
  BNANC(NMe) (5)..(5)
  2'-OMe (6)..(7)
  BNANC(NMe) (8)..(8)
  2'-OMe (9)..(36)
  BNANC(NMe) (37)..(37)
  2'-OMe (38)..(44)
atcctagtagaaaugucaucagacguguaacaaacataagacca

SEQ ID NO: 65 - DNA, 44 bp, artificial sequence
  sense sequence (1)''
  BNANC(NMe) (1)..(1)
  2'-OMe (2)..(40)
  BNANC(NMe) (41)..(41)
  2'-OMe (42)..(44)
taggaucaucaaacaaugugcagacuacuguaaaguauuctggu

SEQ ID NO: 66 - DNA, 44 bp, artificial sequence
  antisense sequence (1)''
  2'-OMe (1)..(4)
  BNANC(NMe) (5)..(5)
  2'-OMe (6)..(36)
  BNANC(NMe) (37)..(37)
  2'-OMe (38)..(44)
aucctaguagaaaugucaucagacguguaacaaacataagacca

SEQ ID NO: 67 - DNA, 40 bp, artificial sequence
  sense sequence (2)''
  2'-OMe (1)..(6)
  BNANC(NMe) (7)..(7)
  2'-OMe (8)..(36)
  BNANC(NMe) (37)..(37)
  2'-OMe (38)..(38)
  BNANC(NMe) (39)..(39)
  2'-OMe (40)..(40)
ggaucatcaaacaaugugcagacuacuguaaaguautctg

SEQ ID NO: 68 - DNA, 40 bp, artificial sequence
  antisense sequence (2)''
  2'-OMe (1)..(2)
  BNANC(NMe) (3)..(3)
  2'-OMe (4)..(5)
  BNANC(NMe) (6)..(6)
  2'-OMe (7)..(34)
  BNANC(NMe) (35)..(35)
  2'-OMe (36)..(40)
cctagtagaaaugucaucagacguguaacaaacataagac

SEQ ID NO: 69 - DNA, 40 bp, artificial sequence
  sense sequence (3)''
  2'-OMe (1)..(6)
  BNANC(NMe) (7)..(7)
  2'-OMe (8)..(38)
  BNANC(NMe) (39)..(39)
  2'-OMe (40)..(40)
ggaucatcaaacaaugugcagacuacuguaaaguauuctg

SEQ ID NO: 70 - DNA, 40 bp, artificial sequence
  antisense sequence (3)''
  2'-OMe (1)..(2)
  BNANC(NMe) (3)..(3)
  2'-OMe (4)..(34)
  BNANC(NMe) (35)..(35)
  2'-OMe (36)..(40)
cctaguagaaaugucaucagacguguaacaaacataagac

SEQ ID NO: 71 - DNA, 36 bp, artificial sequence
  sense sequence (4)''
  2'-OMe (1)..(1)
  BNANC(NMe) (2)..(2)
  2'-OMe (3)..(4)
  BNANC(NMe) (5)..(5)
  2'-OMe (6)..(31)
  BNANC(NMe) (32)..(32)
  2'-OMe (33)..(34)
  BNANC(NMe) (35)..(35)
  2'-OMe (36)..(36)
atcatcaaacaaugugcagacuacuguaaagtautc

SEQ ID NO: 72 - DNA, 36 bp, artificial sequence
  antisense sequence (4)''
  2'-OMe (1)..(3)
  BNANC(NMe) (4)..(4)
  2'-OMe (5)..(32)
  BNANC(NMe) (33)..(33)
  2'-OMe (34)..(36)
uagtagaaaugucaucagacguguaacaaacataag

SEQ ID NO: 73 - DNA, 36 bp, artificial sequence
  sense sequence (5)''
  2'-OMe (1)..(1)
  BNANC(NMe) (2)..(2)
  2'-OMe (3)..(34)
  BNANC(NMe) (35)..(35)
  2'-OMe (36)..(36)
atcaucaaacaaugugcagacuacuguaaaguautc

SEQ ID NO: 74 - DNA, 36 bp, artificial sequence; identical to SEQ ID NO: 72
  antisense sequence (5)''
  2'-OMe (1)..(3)
  BNANC(NMe) (4)..(4)
  2'-OMe (5)..(32)
  BNANC(NMe) (33)..(33)
  2'-OMe (34)..(36)

SEQ ID NO: 75 - DNA, 30 bp, artificial sequence
  psiCHECK2-T200c-3p-s
tcgagtccatcattacccggcagtattagc

SEQ ID NO: 76 - DNA, 30 bp, artificial sequence
  psiCHECK2-T200c-3p-a
ggccgctaatactgccgggtaatgatggac

SEQ ID NO: 77 - DNA, 75 bp, artificial sequence
  psiCHECK2-T199a-3px3-s
tcgagtaaccaatgtgcagactactgtataaccaatgtgcagactactgtataaccaatgtgcagactactgtgc

SEQ ID NO: 78 - DNA, 75 bp, artificial sequence
  psiCHECK2-T199a-3px3-a
ggccgcacagtagtctgcacattggttatacagtagtctgcacattggttatacagtagtctgcacattggttac

SEQ ID NO: 79 - DNA, 29 bp, artificial sequence
  psiCHECK2-T21-5p-s
tcgagtcaacatcagtctgataagctagc

SEQ ID NO: 80 - DNA, 29 bp, artificial sequence
  psiCHECK2-T21-5p-a
ggccgctagcttatcagactgatgttgac